European Patent Application EP 4 621 043 A1, published September 24, 2025. Title: NOVEL MICROORGANISMS, CULTURE OR EXTRACT OF NOVEL MICROORGANISMS, AND METHOD FOR PRODUCING ERGOTHIONEINE. Applicant: KUREHA CORPORATION. The sequence listing filed with the application follows.

SEQUENCE LISTING (14 sequences)

SEQ ID NO: 1 - DNA, 571 bp, Aureobasidium melanogenum
  source 1..571: mol_type = genomic DNA
aaaccaacagggattgccctagtaacggcgagtgaagcggcaacagctcaaatttgaaagctggccttcgggtccgcattgtaatttgtagaggatgctttgggtgaaacgccagtctaagttccttggaacaggacgtcatagagggtgagaatcccgtatgtgactggaaatgttaacctatgtaaagctccttcgacgagtcgagttgtttgggaatgcagctctaaatgggaggtaaatttcttctaaagctaaatattggcgagagaccgatagcgcacaagtagagtgatcgaaagatgaaaagcactttggaaagagagttaaaaagcacgtgaaattgttgaaagggaagcgcttgcaatcagacttgtttaaactgttcggccggtcttctgaccggtttactcagtttggacaggccagcatcagtttcggcggccggataaaggctctgggaatgtggccttcacttcggtgaaggtgttatagcccagggtgtaatacggccagccgggactgaggtccgcgcttcggctaggatgctggcgtaatggttgtaagcgac

SEQ ID NO: 2 - DNA, 563 bp, Aureobasidium melanogenum
  source 1..563: mol_type = genomic DNA
tttccgtaggtgaacctgcggaaggatcattaaagagtaagggtgctcagcgcccgacctccaaccctttgttgttaaaactaccttgttgctttggcgggaccgctcggtctcgagccgctggggattcgtcccaggcgagcgcccgccagagttaaaccaaactcttgttattaaaccggtcgtctgagttaaaattttgaataaatcaaaactttcaacaacggatctcttggttctcgcatcgatgaagaacgcagcgaaatgcgataagtaatgtgaattgcagaattcagtgaatcatcgaatctttgaacgcacattgcgccccttggtattccgaggggcatgcctgttcgagcgtcattacaccactcaagctatgcttggtattgggtgccgtccttagttgggcgcgccttaaagacctcggcgaggcctcaccggctttaggcgtagtagaatttattcgaacgtctgtcaaaggagaggacttctgccgactgaaacctttatttttctaggttgacctcggatcaggtagggatacccgctgaacttaa

SEQ ID NO: 3 - DNA, 605 bp, Ustilago sp.
  source 1..605: mol_type = genomic DNA
aaactaacaaggattcccctagtaacggcgagtgaagagggaagagcccaagattgaaagctggcgtcttcggcgtccgcattgtaatctcaagaagtgttttccgcttcggaccatgcctaagtcccttggaaaagggcatcatagagggtgataatcccgtacatggcatggagcgcccgaggctttgtgatacgctttctaagagtcgagttgtttgggaatgcagctcaaaatgggtggtaaatgccatctaaggctaaatattggggagagaccgatagcgaacaagtacagtgatggaaagatgaaaagaactttgaaaagagagttaaacagtacgtgaaattgccaaaagggaagggtaggaggtcagagatgcgttctgggattcagccttgcttttgcttggtgtttttcccagattgcaggccaacgtcggttttgggcgctggagaagggtggaaggaatgtggcacccctcggggtgtgttatagccttctactggatacagtgaccgagaccgaggacagcagcgtactcgcaagagcgggccttcgggcacctttacgcttagggcgttggcataatggccctctaccac

SEQ ID NO: 4 - DNA, 730 bp, Ustilago sp.
  source 1..730: mol_type = genomic DNA
tatctgtaggtgaacctgcagatggatcatttcgatgaaaaccttttttcttgaggtgtggctcgcacctgtctaactaaaattgagctaccttttttcaacacggttgcatcggttggcctgtcaaacagtgcggcgacgagaatttattttcttcgagccaagctaggcgacggaccgacacttaatcaacacttttgatgatctaggatttgaacgtataaaagttacttttttaataactaaaaaacaacttttggcaacggatctcttggttctcccatcgatgaagaacgcagcgaattgcgataagtaatgtgaattgcagaagtgaatcatcgaatctttgaacgcaccttgcgctcccggcagatctaatctggggagcatgcctgtttgagggccgcgaattgtttcgaacgacagcttttttcacgaaaagttggcggatcggtattgagggttttttgccatttaccatggctccctcgaaatgcattagcgcatccatttgataggcaagacggacgaaagctcgattttcgctctctcttccctgccgggttttgataatatcaggacttcggagaggttgagatgggtaagagctggacgcaacgacttgctgtttggagtgcttctgaaacccgcccatgccaaggacttgttccttggaagggattttataattcatcggcctcagattggtaggactacccgctgaacttaa

SEQ ID NO: 5 - DNA, 605 bp, Dirkmeia churashimaensis
  source 1..605: mol_type = genomic DNA
aaactaacaaggattcccctagtaacggcgagtgaagagggaagagcccaagattgaaagctggcgtcttcggcgtccgcattgtaatctcaagaagtgttttccgcttcggaccatgcctaagtcccttggaaaagggcatcatagagggtgataatcccgtacatggcatggagcgcccgaagctttgtgatacgctttctaagagtcgagttgtttgggaatgcagctcaaaatgggtggtaaatgccatctaaggctaaatattggggagagaccgatagcgaacaagtacagtgatggaaagatgaaaagaactttgaaaagagagttaaacagtacgtgaaattgccaaaagggaagggtaggaggtcagagatgcggcctgggattcagccttgcttttgcttggtgtttttcccagattgcaggccaacgtcggttttgggcactggagaagggtaggaggaacgtggcacctctcggggtgtgttatagcctcctactggatacagcgaccgagaccgaggacagcagcgtactcgcaagagcgggccttcgggcacctttacgcttagggcgttggcataatggccctctaccac

SEQ ID NO: 6 - DNA, 732 bp, Dirkmeia churashimaensis
  source 1..732: mol_type = genomic DNA
tatctgtaggtgaacctgcagatggatcatttcgatgaaaaccttttttctgaggtgtggctcgcacctgtctaactaaacttgagctacccaattttcaacacggttgcatcggttagctgtcaaacagtgcggaaacgcgttgtgcgacggttgacacaaacacaaacacttttgatgatctaggatttgaatgaaagttcatttttatgatggaaccgactggtaatgcggtcgtctaaatctaaaaaacaacttttggcaacggatctcttggttctcccatcgatgaagaacgcagcgaattgcgataagtaatgtgaattgcagaagtgaatcatcgaatctttgaacgcaccttgcgctcccggcagatctaatctggggagcatgcctgtttgagggccgcgaattgtttcgaacgacagcttttttcttgtagaagagttggcggatcggtagtgagggtctttgccatttaccgtggctccctcgaaatacattagcgcatccatttaataggcaagacggacgaaagctcgattttcgccccctcttccctgccgggttttgataatatcaggacttcggagagcggagagaagggtgagagctggacgcgacgttttgctggttggagtgcttctgaaccccgcccatgcctttcgcaagaaaggaagggatttttcaattcatcggcctcagattggtaggactacccgctgaacttaa

SEQ ID NO: 7 - DNA, 605 bp, Dirkmeia churashimaensis; identical to SEQ ID NO: 5
  source 1..605: mol_type = genomic DNA

SEQ ID NO: 8 - DNA, 732 bp, Dirkmeia churashimaensis; identical to SEQ ID NO: 6
  source 1..732: mol_type = genomic DNA

SEQ ID NO: 9 - DNA, 605 bp, Dirkmeia churashimaensis; identical to SEQ ID NO: 5
  source 1..605: mol_type = genomic DNA

SEQ ID NO: 10 - DNA, 732 bp, Dirkmeia churashimaensis; identical to SEQ ID NO: 6
  source 1..732: mol_type = genomic DNA

SEQ ID NO: 11 - DNA, 605 bp, Dirkmeia churashimaensis; identical to SEQ ID NO: 5
  source 1..605: mol_type = genomic DNA

SEQ ID NO: 12 - DNA, 731 bp, Dirkmeia churashimaensis
  source 1..731: mol_type = genomic DNA
tatctgtaggtgaacctgcagatggatcatttcgatgaaaccttttttctgaggtgtggctcgcacctgtctaactaaacttgagctacccaattttcaacacggttgcatcggttagctgtcaaacagtgcggaaacgcgttgtgcgacggttgacacaaacacaaacacttttgatgatctaggatttgaatgaaagttcatttttatgatggaaccgactggtaatgcggtcgtctaaatctaaaaaacaacttttggcaacggatctcttggttctcccatcgatgaagaacgcagcgaattgcgataagtaatgtgaattgcagaagtgaatcatcgaatctttgaacgcaccttgcgctcccggcagatctaatctggggagcatgcctgtttgagggccgcgaattgtttcgaacgacagcttttttcttgtagaagagttggcggatcggtagtgagggtctttgccatttaccgtggctccctcgaaatacattagcgcatccatttaataggcaagacggacgaaagctcgattttcgccccctcttccctgccgggttttgataatatcaggacttcggagagcggagagaagggtgagagctggacgcgacgttttgctggttggagtgcttctgaaccccgcccatgcctttcgcaagaaaggaagggatttttcaattcatcggcctcagattggtaggactacccgctgaacttaa

SEQ ID NO: 13 - DNA, 605 bp, Dirkmeia churashimaensis; identical to SEQ ID NO: 5
  source 1..605: mol_type = genomic DNA

SEQ ID NO: 14 - DNA, 732 bp, Dirkmeia churashimaensis; identical to SEQ ID NO: 6
  source 1..732: mol_type = genomic DNA